European Patent Application EP 4 159 756 A1, published April 5, 2023. Title: Anti RNA virion antibody of HBV. Applicant: RCMG. The sequence listing filed with the application follows.

SEQUENCE LISTING (19 sequences)

SEQ ID NO: 1 - protein, 184 aa, Unknown
  none
MGWRWILLFLLSGTAGVHCQVQLQQSGPELVKPGALVKISCKASGYTFTSYDINWVKQRPGQGLEWIGWIYPGDGRTKYNEKFKGKATLTADKSSSTAYMQLSSLTSENSAVYFCVRSHDSNYGAWFPYWGQGTLVTVSAAKTTPPSVYPLAPGSAAQTNSMVTLGCLVKGYFPEPVTVTWNSG

SEQ ID NO: 2 - protein, 150 aa, Unknown
  none
MKLPVRLLVLMFWIPASRSDVLMTQTPLSLPVSLGNQASISCRSSQNIVHSNGNTYLEWYLQKPGQSPKLLIYKVSNRFSGVPDRFSGSGSGTDFTLKISRVEAEDLGVYYCFQGSHVPLTFGTGTKLELKRADAAPTVSIFPPSSEQLT

SEQ ID NO: 3 - protein, 131 aa, Unknown
  none
MKVLSLLHLLTAIPGILSDVQLQESGPGLVKPSQSLSLTCSVTGYSITSTYYWNWIRQFPGNKLEWMGYISYDGSTNYHPSLKNRISITRDTSKNQFFLKLNSVTAEDTATYYCSRGITYYWGQGTTLTVS

SEQ ID NO: 4 - protein, 131 aa, Unknown
  none
MKLPVRLLVLMFWIPASSSDVVMTQTPLSLPVSLGDQASISCRSSQSLIHSNGNTYLHWYLQKPGQSPNLLIYKVSNRFSGVPDRFSGSGSGTDFTLKISRVEAEDLGVYFCFQSTHIPHTFGGGTKLEIK

SEQ ID NO: 5 - protein, 138 aa, Unknown
  none
MYLGLNCVFIVFLLKGVQSEVKLEESGGGLVQPGGSMKFTCVASGFTFSNYWMNWVRRSPEKGLEWVAEIRLKSDNYATHYAESVKGRFTISRDDSKSSVYLQMNNLRGEDTAIYYCTSPTSGTPFAYWGQGTLVIVS

SEQ ID NO: 6 - protein, 133 aa, Unknown
  none
MDSQAQVLMLLLLWVSGTCGDIVMSQSPSSLPVSVGEKVTMSCRSSQSLLYSNNQKNYLAWYQQKPGQSPKLLIYWASTRESGVPDRFTGSGSGTDFTLTISSVKAEDLAIYYCQQYYTYPWTFGGGTKLEIK

SEQ ID NO: 7 - protein, 138 aa, Unknown
  none
MYLGLNCVFIVFLLKGVQSEVNLEESGGGLVQPGGSMKLSCVASGFTFNNYWMNWVRQSPEKGLEWVAEIRVESNDYATHYAESVKGRFTISRDDSKSSVYLQMNNLRAEDTGIYYCTSPTAGTPFAYWGQGILVTVS

SEQ ID NO: 8 - protein, 127 aa, Unknown
  none
MESHTQAFVFAFLWLSGVDGDIVMTQSQKFMSTSVGDRVSITCKASQNVGTAVAWYQQKPGQSPKLLIYSASNRYTGVPDRFTGSGSGTDFTLTISNMQSEDLADYFCQQYSSYPYTFGGGTKLEIK

SEQ ID NO: 9 - DNA, 552 bp, Unknown
  none
atgggatggagatggatccttcttttcctcctgtcaggaactgcaggtgtccactgccaggttcagctgcagcagtccggacctgagctggtgaagcctggggctttagtgaagatatcgtgcaaggcttctggttacaccttcacaagctacgatataaactgggtgaagcagaggcctggacagggacttgagtggattggatggatttatcctggagatggtcgtactaagtacaatgagaaattcaagggcaaggccacactgactgcagacaaatcctccagcacagcctatatgcagctcagcagcctgacttctgagaactctgcagtctatttttgtgtaagatcacacgatagtaattacggggcctggtttccttactggggccaagggactctggtcactgtctctgcagccaaaacgacacccccatctgtctatccactggcccctggatctgctgcccaaactaactccatggtgaccctgggatgcctggtcaagggctatttccctgagccagtgacagtgacctggaactctgga

SEQ ID NO: 10 - DNA, 450 bp, Unknown
  none
atgaagttgcctgttaggctgttggtgctgatgttctggattcctgcttccagaagtgatgtattgatgacccaaactccactctccctgcctgtcagtcttggaaatcaagcctccatctcttgcagatctagtcagaacattgtacatagtaatggaaacacctatttagaatggtacctgcagaaaccaggccagtctccaaagctcctgatctacaaagtttctaaccgattttctggggtccccgacaggttcagtggcagtggatcagggacagatttcacactcaagatcagcagagtggaggctgaggatctgggagtttattactgctttcaaggttcacatgttccgctcacgttcggtactgggaccaagctggagctgaaacgggctgatgctgcaccaactgtatccatcttcccaccatccagtgagcagttaaca

SEQ ID NO: 11 - DNA, 393 bp, Unknown
  none
atgaaagtgttgagtctgttgcacctgttgacagccattcctggtatcctgtctgatgtacagcttcaggagtcaggacctggcctcgtgaaaccttctcagtctctgtctctcacctgctctgtcactggctactccatcaccagtacttattactggaactggatccggcagtttccaggaaacaaactggaatggatgggctacataagctacgacggtagcactaattatcatccatctctcaaaaatcgcatctccatcactcgtgacacatctaagaaccagtttttcctgaagttgaattctgtgactgctgaggacacagctacatattactgttcaagagggattacctactactggggccaaggcaccactctcacagtctcc

SEQ ID NO: 12 - DNA, 393 bp, Unknown
  none
atgaagttgcctgttaggctgttggtgctgatgttctggattcctgcttccagcagtgatgttgtgatgacccaaactccactctccctgcctgtcagtcttggagatcaagcctccatctcttgcagatctagtcagagccttatacacagtaatggaaacacctatttacattggtatctgcagaagccaggccagtctccaaacctcctgatctacaaagtttccaaccgattttctggggtcccagacaggttcagtggcagtggatcagggacagatttcacactcaagatcagcagagtggaggctgaggatctgggagtttatttctgttttcaaagtacacatattcctcacacgttcggaggggggaccaagctggaaataaaa

SEQ ID NO: 13 - DNA, 414 bp, Unknown
  none
atgtacttgggactgaactgtgtattcatagtttttctcttaaaaggtgtccagagtgaagtgaagcttgaggagtctggaggaggcttggtgcaacctggaggatccatgaaattcacctgtgttgcctctggatttactttcagtaattactggatgaactgggtccgccggtctccagagaaggggcttgagtgggttgctgaaattagattgaaatctgataattatgcaacacattatgcggagtctgtgaaagggaggttcaccatctcaagagatgattccaaaagtagtgtctacctgcaaatgaacaacttaagaggtgaagacactgccatttattactgtaccagccctacaagtgggacgccgtttgcttactggggccaagggactctggtcattgtctct

SEQ ID NO: 14 - DNA, 399 bp, Unknown
  none
atggattcacaggcccaggttcttatgttactgctgctatgggtatctggtacctgtggggacattgtgatgtcacagtctccatcctccctacctgtgtcagttggagagaaggttactatgagctgcaggtccagtcagagccttttatatagtaacaatcaaaagaactacttggcctggtaccagcagaaaccagggcagtctcctaaactgctgatttactgggcatccactagggaatctggggtccctgatcgcttcacaggcagtggatctgggacagatttcactctcaccatcagcagtgtgaaggctgaagacctggcaatttattactgtcagcaatattatacctatccgtggacgttcggtggaggcaccaagctggaaatcaaa

SEQ ID NO: 15 - DNA, 414 bp, Unknown
  none
atgtacttgggactgaactgtgtattcatagtttttctcttaaaaggtgtccagagtgaagtgaaccttgaggagtctggaggaggcttggtgcaacctggaggatccatgaaactctcctgtgttgcctctggattcactttcaataattattggatgaactgggtccgccagtctccagagaaggggcttgagtgggttgctgaaattagagtggaatctaatgattatgcgacacattatgcggagtctgtgaaagggaggttcaccatctcaagagatgattccaaaagtagtgtctacctccaaatgaacaacttaagagctgaagacactggcatttattactgtaccagtcctacagctgggacgccgtttgcttactggggccaagggattctggtcactgtctct

SEQ ID NO: 16 - DNA, 381 bp, Unknown
  none
atggagtctcatactcaggcctttgtattcgcgtttctctggttgtctggtgttgatggagacattgtgatgacccagtctcaaaaattcatgtccacatcagtaggagacagggtcagcatcacctgcaaggccagtcagaatgtgggtactgctgtagcctggtatcaacagaaaccaggacaatctcctaaactactgatttactcggcatccaatcggtacactggagtccctgatcgcttcacaggcagtggatctgggacagatttcactctcaccatcagcaatatgcagtctgaagacctggcagattatttctgccagcaatatagcagctatccgtacacgttcggaggggggaccaagctggaaataaaa

SEQ ID NO: 17 - DNA, 43 bp, Artificial Sequence
  none
gacgttgtaaaacgacggccaggcctcaaggtcggtcgttgac

SEQ ID NO: 18 - DNA, 20 bp, Artificial Sequence
  none
ctgtgccttctcatctgccg

SEQ ID NO: 19 - DNA, 22 bp, Artificial Sequence
  none
gacgttgtaaaacgacggccag